European Patent Specification EP 2 655 629 B1, published April 24, 2024. Title: Brassica plant comprising a mutant ALCATRAZ allele. Applicant: Bayer BioScience N.V. Laga, Benjamin. The sequence listing filed with the application follows.

SEQUENCE LISTING (20 sequences)

SEQ ID NO: 1 - DNA, 2547 bp, Brassica napus
acgaaaaccaccatcgtccgattcatcatccgtcaactttggcccactgggtttggacacaagtgcgtcgtactgcggctgttccagtttaatgtcgaagtcgaagatgggtagttcccaccacagtttctgccatcttcatccgacaaactctttagcattctccggcaaattctgtcacgtactccgacaacccaaccttccccacccaagagaaacatttcatccgctgagatgttcgactggaactttcctttcgttttcggcggagcagtttctagcgcaggctatgcggtcattgaaactgggggagacaaatgtgcttttgagaacaaggtaaaacttaacaactttattgctgtcgtcaaattataatcgctttgtttaaagaaatactaaagagagcatctctctcgtctctctcatcttttcttgaagtttccagcttttggatttgcagtctctggccaacgtccggttcgccggcgttgtgtcttgtaaatttgtaattagttttttttttgttttgtcaccgacttgtttggggtttgtctccggttttaatccggttttgttcttccgtcttgtacggatcttaactccgattgggttcggtttatcttttgtttaatcggcttaaaatctctagcctttgtgtgttctaatctctttctggttttctccaatcgattgaacagatttgggttttcactaatgcttgactctttgctcatgagaaaataaaccctcacttcttggctatggcgatttaaagtgcaggtcatccatgtgtgaagattcaaggtgttgcgattatccggagaagagtgaagatttaaaactctggtcgtgttcagacggtgttttaaagaatgctccaatccgattaactgggttcttaactcttggtgtttaagtctaaatctcaacaatcttttgggataatcaaagcaaaggcttcaaacgatgcaaataaaaaaactaagcttgctcacaacaaaacgtttgatcaaaagagaaagcactgtggtggctcaagtcttcggtggaggtagaaacctcttctggttctcagagaaggtgcgtgtttggcttggaaggagatagatgtatatcggagcgattgcttcattgtcggtcgattgtcgccgtcttgatcgtgattgtcatggatttggagtggttattatccagctaccggctgtgtgaataagacgtttccgggaaacctttataggcttcgccgtggggtgatggtgcgtatgaggcgcggggagagcacactcaaggtccaatggagagacttagttgggattgaagggtgtttacagcgacggttaaggattctaacctctctcgattcagtttatatgtttggtgatgttcgtgtgcgtctagtctatctcgatgctcctctcattttgtgttaattgttgatgagttctatttcggtaagctcgtctttgagcgcaaggtggagcactcctctactgaagttctgttttactctcatgcttctcgacatcttttttcttcgtgtctttgttagttttttaagggtttgtgttgtatccatcttttggctccgggtggtaaatgttaccgcgccggcttatggttttggaaggaatgtattccttgccggctctggtttgtaagaaatgttgtttttgtgtttaatataatctacagatgacaaaaaaaaaaaaaaaataactaaagagagagaaatggagtcactaaagaacaccatttttctttgtaatggtaacaataacactcaatagaaatggagtcagacagcgaaactcgttgaagagaaacattgatacacagttccacaacttgtctgaaaaggtttctgtctttttccttttaaatattcttgatctgtaaaaattaaaaaaataataaatagaatccgaaaatattgcagaggagaaggagcaagatcaacgagaaaatgaaagctttgcagaaaatgaaagctttgcagaagcggatactcaattccaacaagttaaattgaatgttccaatctttatacttcagatctctatcttgagaatgagaaacattgttttttttttatagttgtagacagataaagtctccatgctttgatgaagcaatagaatatctgaagctgcttcaacttcaagtgcaggtttcttactaaagatcatatataatcaaagtctaatctgtaaaacatatcatctgattaacttatttactccataaagcagactttagccgttatgaatggtctaggcctaaaccctcagcgactaccaccagttctaccgcctacgcagacaaggatcaatggaaccttagaacaagacctcaactttgggactctgcttggtgcttctcactcgctggttaaccgtgaaccacccgaatcaactcaggaaatgtgcttttccacagacactctgctttgaagacaacattcagacgtgaagatgattcgaagtcaagatctcctctgagtaccgtataccacaaatggctgggcacaaggcgagtactcgttatttt

SEQ ID NO: 2 - DNA, 1415 bp, Brassica napus
ggttgagctcagtccactagcttatcgagctgatctagtttcaatgagcttgtccaacatactgctcgaccagttccccagctcgcctagctcgtccagctctttacactcttccttagctcggtccagcttcttttcttcgtttttctcctttttcttggctaaatccggatcattcctaagacttaaccttttgttcagaccatggaacgcttgtcttaaagtttttcgactggcttgcacgttccctcgtcccatggcccgttccaacgatccttagcaaagatcggggatgctacaattacaaatagaatagaaagggagatatttattgattttcgaagaaacacatataaacatatagaattattctatttgttattattgtatttttacataagcaataaaaatttgattgaaaaactaatagaggctaagaatatttatatctccataccacctcgaagtccaaaatactattcaaaagatccaataaattgccgacaaaaaaaaagatccaataaatcaatggtaacaacttttgttgccgttaaactacactcgctttgtttaaagaacaaaaacaaaactaacttttgtttttcttttgcaatggtaacaataacactaaagagaaacggagccaggtagcgaaactcgttgaagagaaacattgatgcacagttccacaacttgtctgaaaaggcttccgtctttcagcttttttaaatattcttgatctgaaaaatatataaaaaaacaataatagaatcagaaaatattgcagagaaggaggagcaagatcaacgagaaaatgaaatctttgcagaagctgatacccaattccaacaaggtaaattgaaagtttgaattttcatccttcagaacttagacatgataaacattctttttatatatatatatatatatatatatttgtagacagataaagcctcaatgcttgatgaagctatagaatatctgaagcagcttcaacttcaagtgcaggttttttattttattttattttacttactaagatcctttatatgcaatcaaagtttaaatttgtaaaccccattgtctgattaacataatcactgcataatacagactttagctgttatgaatggtttaggcctaaactctatgcgactaccaccagttctaccgtctacgcagacaaggttcaaatggaaccttacaacaagagcagcactttgggactcggcttggtgctcctcactcgatggttaaccgtgaaccaccccaagcaactcaggaaatgtgcttttccacaggcacgctgctttgaagacaaagatgattcgaagtcaacatctccggcttagtacactaccaaacagtagtcaaaactgtttttagtctagtatttgcatactccaaagttcagt

SEQ ID NO: 3 - DNA, 1201 bp, Brassica napus
  variation (668)..(668): G to A in ALC-GR3-EMS07
gattatggctagagtgatttgccacgcgcctgcctatttattatgaaaagcctcagtaactctgtgacgagaagaattcacagagagagagaggagagagatgggtaattccgacgaaggtggtcgtcttcctgctccatcttcttcagacgaactctcgagcattctgcggcaggtactgtcccgtactcccacagctcaaccttctttctcaccgaagaaaatcgtttcctccgctgagatgttcaaccgaacattccccctcgttcccggcggagcggtttcttacgccgcttgtgcagccgctgaaactggggaaagcaaatgtggtttcgaaaacaaggtaaacttaacgatgttagttgccgtgaaagtaccctcgcttttgattaaagaaaaaataacttagttgttgtttttgcttggtaatggttaacacaacactaaagagaaatggagctagacagcgaaattcattgaagagaaacattgatgcacagttccacaacttgtctgaaaaggtttcgtctttatccttttaagattcttgatttggtttaaaaaaaactagagataataatagaaactggatatattgcagaggaggaggagcaagatcaatgagaaaatgaaagcattgcagaaactgatacccaattccaacaaggtaaatataaagttcgacattttatccttcagaactgagtgtcgtgaaaagcatttattttgtttttttatgtttggtagacagataaggcctcaatgcttgatgaagctatagaatatctgaaacagcttcaacttcagtttcaggttctttttctatatgttccttacgctatgatcataaacaactaaatttgtaaaaccaaacatctgattaacttttaatgactgcagacgttagccgctatgaatggtttaggcctaaatcctctgcgattaccaccaattctaccgcctacgcagacaaggatcactggaacctctgaacaagggctgaaccttgagactctgcttggtggttctcactcgatggctaaccatgaaccacccgaaccaactcaggaaatgtgcttttccacaaccactctgctttgaagacaacgttcaaagagtgaagaggattcgaagtcagatttcctctctccacagaaacatgagccgaaaatgatttgtagagtctagtatttggttatat

SEQ ID NO: 4 - DNA, 1207 bp, Brassica napus
  variation (646)..(646): C to T in ALC-GR4-EMS04
ccagattatgtctagagtgatttgccacgcgcctgcctatttattatgaaaagcctcagtaacttgtgatgagaagaattcacagagagagaggagagagatgggtaattccgatgaaggtgatcgtcttcctgctccatcttcttcggacgaactctcgagcattctccggcaggtactgtcccgtactcccacagctcaaccttctttctcaccgaagaaaatcgtttcctccgctgagatgttcaaccgaaccttccccctcgttcccggcggagcggtttcttacgccgcttgtgcagtcgctgaaactggggaaggcaaatgtggtttcgaaaacaaggtaaacttaacgatgttagttgccgtgaaactattaccctcgcttgttgattaaagaaaaaaataactttattgtgtttttggttggtaatggttaaaaaacactaaagagaaatggagctagacagcgaaattcattgaagagaaacattgatgcacagttccacaccttgtctgaaaaggttttgtctttatccttttaagattcttgatttggtttaaaaaaaaaactagagataataatagaaactggatatattgcagaggaggaggagcaagatcaacgagaaaatgaaagctttgcagaaactgatacccaattccaacaaggtggtaaataccaagttcgactttttatctttcagaactcagttgtgagatacatttgttttgtttttttttatgttttgtagacagaaaaggcctcaatgcttgatgaagctatagaatatctgaaacagcttcaacttcagtttcaggttctttttctatatgttccttacgctatgatcataaacaactaaatttgtaaacccaaacatctgattaacttgatgaatgcagacgttagccgctatgaatggtttaggcctaaatcctctgcgattaccaccaattctaccgcctacgcagacagggatcactggaacctcagaacaagggctgaaccttgagactctgcttggtggttctcactcgatggctaaccttgaaccacccgaaccaactcaggaaatgtgctttcccacaaccactctgctttgaagacaacgttcagacagtgaagaggattcgaagtcagatttcctctccacagaaacatgagccgaaaatgatttggttatatttcaaagtgttatgctaa

SEQ ID NO: 5 - DNA, 1174 bp, Brassica napus
gctcataaatcacgcgcgtacttccccacctatttattatgaaaagcctcagtaaactagtaaagtgaattgtgaaggattacagagagacagagagagatgggtaattccgacgccagagatcgtcttcctgctccatcttcttcagacgaactctcgagcattctccggcaggtactttcccgtactcctccgactgctcaaccttctttctcacggaagaaaatcgtttcctccggtgagatgttcaaccgaacgttccctctcgttcacggcggagcggtttcttacgccgcttgtgcagtctctgaaactgaggaaggaaaatgtgctttcgagaaccaggtaaacttaacaatgttagttgccgtgaaactacactcgctttggttaaagaacaaaaaaaaaacttgttgttgtttttgctttgtaatggtaaaacaacactaaatagaaatggagctagacagcgaaattgatgcacagttccacaacttgtttgaaaaggtttctgtctttatccttttaacattctttgaattgattttttttttaaagaactggacataataatagttaatagaaactgaaagtattgcagataggaggagcaagatcaacgagaaaattaaagctttacagaaactgatacccaattccaacaaggtatatagcaagttcgactttttatccctcagaactcagttgtgagaagcatttgttttgttttttatggtatgtagacagataaggcctcaatgtttgatgaaactatagaatatttgaaacagcttcaacttcagttttcaactttgggtttcgggcaagcgcactaaggggttgattggtaagtgctatcatttcattttttgactgtagaaatattgctgtggtttttattgctttggctttagatttttaatttttaaaagtctttaaatatgggctgtaggtttttgtctctgcagagaaattgtaaagacataatttcaaagaagtgctgtggattttataaaaagactgtgaacttaaaaaaaaatagaaatcaagattggtgtagatttagtgttctagaaagaaatgaggctgtagagagcactcatcactaccaatcacaccctaaaaagagttatgttccctaataagaaaaaaggaaagcggttacgcgtaaaat

SEQ ID NO: 6 - DNA, 1360 bp, Brassica napus
ccccaagcctcctcatgccgtctggacacaagtgcgtcgtactgtggctgttccagtttaatgtcgaagtcgaagatgggtagttccgacgacagtttctgccatcttcatccgacaaactctctagcattctccggcagattctgtcacgtactccgacaacccaaccttccccacccaagagaaacatttcctccgctgagatgtttgactgaaactttcctttcgatttcagtggagcagtttctagcgcaggctatgaggtcattgaaattggaggagacaaatgtgcttttgagaacaaggtaaaacgtgttaaaaaaaagaacaaggtaaaacttaacaactttagttgctgtcgtccaattttttttttttgaattagctagaggtatcctgaccccacagaagtgatccagactagtcatgtgttgccacatgtcggtcctctatccctggcaatgctgaaatgttaattctccagtggctgggattcgaacccagctgtcgtcaaattataatcggttggtttaaagaaatactaaagagagagaaatggagtcactaaagaacaccatttttctttgaaatggtaacaataaaactcaatagaaatggagtcagacagtaaaacttgttgaagagaaacattgatacacagttccacaacttgtctgaaaaggtttctgtctttttccttttaaatattcatgatctgtaaaaattaaaaaattaataaatagattccgaaaatatttcagaggagaaggagcaagatcaacgagaaaatgaaagctttacagaagctgatactcaattccaacaagttaaattgaatgttccaatctttatacttcagatctctatcttgagaatgagaaacattgttttgttttttaatagttgtagacatataaagtctcattgctttgatgaagcgataaaatatctgacgctgcttcaacttcaagtgcaggtttcttactaaagatcatatataatcaaagtctaatctgtaaaacatatcatctgattaacttatttactccataatgcagactttagccgttatgaatggtctaggcctaaaccctcagcgactaccaccagttctaccgcctacgcagacaaggatcaatggaaccttagaacaagacctcaactttgggactctgcttggtgcttctcactcgctggttaaccggtgaaccacctgaatcaactcaggaaatgtgcttttccacagacactctgctttgaagacaacattcggacgtgaagatgattcgaagtcaagatctcctcttagtaccgtataccacaaagagcttgtgagctttggtcttcatcagttgggctg

SEQ ID NO: 7 - DNA, 648 bp, Brassica napus
atgggtaattccgacgaaggtggtcgtcttcctgctccatcttcttcagacgaactctcgagcattctgcggcaggtactgtcccgtactcccacagctcaaccttctttctcaccgaagaaaatcgtttcctccgctgagatgttcaaccgaacattccccctcgttcccggcggagcggtttcttacgccgcttgtgcagccgctgaaactggggaaagcaaatgtggtttcgaaaacaagagaaatggagctagacagcgaaattcattgaagagaaacattgatgcacagttccacaacttgtctgaaaagaggaggaggagcaagatcaatgagaaaatgaaagcattgcagaaactgatacccaattccaacaagacagataaggcctcaatgcttgatgaagctatagaatatctgaaacagcttcaacttcagtttcagacgttagccgctatgaatggtttaggcctaaatcctctgcgattaccaccaattctaccgcctacgcagacaaggatcactggaacctctgaacaagggctgaaccttgagactctgcttggtggttctcactcgatggctaaccatgaaccacccgaaccaactcaggaaatgtgcttttccacaaccactctgctttga

SEQ ID NO: 8 - DNA, 648 bp, Brassica napus
atgggtaattccgatgaaggtgatcgtcttcctgctccatcttcttcggacgaactctcgagcattctccggcaggtactgtcccgtactcccacagctcaaccttctttctcaccgaagaaaatcgtttcctccgctgagatgttcaaccgaaccttccccctcgttcccggcggagcggtttcttacgccgcttgtgcagtcgctgaaactggggaaggcaaatgtggtttcgaaaacaagagaaatggagctagacagcgaaattcattgaagagaaacattgatgcacagttccacaccttgtctgaaaagaggaggaggagcaagatcaacgagaaaatgaaagctttgcagaaactgatacccaattccaacaagacagaaaaggcctcaatgcttgatgaagctatagaatatctgaaacagcttcaacttcagtttcagacgttagccgctatgaatggtttaggcctaaatcctctgcgattaccaccaattctaccgcctacgcagacagggatcactggaacctcagaacaagggctgaaccttgagactctgcttggtggttctcactcgatggctaaccttgaaccacccgaaccaactcaggaaatgtgctttcccacaaccactctgctttga

SEQ ID NO: 9 - protein, 215 aa, Brassica napus
  bHLH domain (91)..(142)
  bHLH domain (92)..(142)
MGNSDEGGRLPAPSSSDELSSILRQVLSRTPTAQPSFSPKKIVSSAEMFNRTFPLVPGGAVSYAACAAAETGESKCGFENKRNGARQRNSLKRNIDAQFHNLSEKRRRSKINEKMKALQKLIPNSNKTDKASMLDEAIEYLKQLQLQFQTLAAMNGLGLNPLRLPPILPPTQTRITGTSEQGLNLETLLGGSHSMANHEPPEPTQEMCFSTTTLL

SEQ ID NO: 10 - protein, 215 aa, Brassica napus
  bHLH domain (92)..(142)
MGNSDEGDRLPAPSSSDELSSILRQVLSRTPTAQPSFSPKKIVSSAEMFNRTFPLVPGGAVSYAACAVAETGEGKCGFENKRNGARQRNSLKRNIDAQFHTLSEKRRRSKINEKMKALQKLIPNSNKTEKASMLDEAIEYLKQLQLQFQTLAAMNGLGLNPLRLPPILPPTQTGITGTSEQGLNLETLLGGSHSMANLEPPEPTQEMCFPTTTLL

SEQ ID NO: 11 - DNA, 22 bp, Artificial
  primer
aggaggaggagcaagatcaatg

SEQ ID NO: 12 - DNA, 26 bp, Artificial
  primer
aacaaaataaatgcttttcacgacac

SEQ ID NO: 13 - DNA, 24 bp, Artificial
  probe
tcgaactttatatttatcttgttg

SEQ ID NO: 14 - DNA, 23 bp, Artificial
  probe
cgaactttatatttatcttgttg

SEQ ID NO: 15 - DNA, 23 bp, Artificial
  probe
tgtcgaactttatatttaccttg

SEQ ID NO: 16 - DNA, 23 bp, Artificial
  primer
agaggaggaggagcaagatcaac

SEQ ID NO: 17 - DNA, 30 bp, Artificial
  primer
aaagataaaaagtcgaacttggtatttacc

SEQ ID NO: 18 - DNA, 16 bp, Artificial
  probe
agctttgtagaaactg

SEQ ID NO: 19 - DNA, 16 bp, Artificial
  probe
aaagctttgcagaaac

SEQ ID NO: 20 - DNA, 508 bp, Brassica napus
agatgggtaattccgatgaaggtgatcgtcttcctgctccatcttcttcggacgaactctcgagcattctccggcaggtactgtcccgtactcccacagctcaaccttctttctcaccgaagaaaatcgtttcctccgctgagatgttcaaccgaaccttccccctcgttcccggcggagcggtttcttacgccgcttgtgcagtcgctgaaactggggaaggcaaatgtggtttcgaaaacaaggtaaacttaacgatgttagttgccgtgaaactaccctcgcttgttgattaaagaaaaaaataactttattgtgtttttggttggtaatggttaaaaaacactaaagagaaatggagctagacagcgaaattcattgaagagaaacattgatgcacagttccacaccttgtctgaaaaggttttgtctttatccttttaagattcttgatttggtttaaaaaaaaaactagagataataatagaaactggatatattgcagagg